European Patent Application EP 4 417 212 A2, published August 21, 2024. Title: TRANSPLANT TOLERANCE INDUCTION WITH CARBODIIMIDE TREATED TOLERIZING VACCINE. Applicant: REGENTS OF THE UNIVERSITY OF MINNESOTA. The sequence listing filed with the application follows.

SEQUENCE LISTING (47 sequences)

SEQ ID NO: 1 - protein, 15 aa, synthetic construct
  REGION 1..15: note = Description of Artificial Sequence: Syntheticpeptide
LSSPLALAGDTRPRF

SEQ ID NO: 2 - protein, 15 aa, synthetic construct
  REGION 1..15: note = Description of Artificial Sequence: Syntheticpeptide
VLTVTLMVLSSPLAL

SEQ ID NO: 3 - protein, 15 aa, synthetic construct
  REGION 1..15: note = Description of Artificial Sequence: Syntheticpeptide
WTFQTLVMLETVPRS

SEQ ID NO: 4 - protein, 15 aa, synthetic construct
  REGION 1..15: note = Description of Artificial Sequence: Syntheticpeptide
QHHNLLVCSVSGFYP

SEQ ID NO: 5 - protein, 15 aa, synthetic construct
  REGION 1..15: note = Description of Artificial Sequence: Syntheticpeptide
NVRFDSDVGEFRAVT

SEQ ID NO: 6 - protein, 15 aa, synthetic construct
  REGION 1..15: note = Description of Artificial Sequence: Syntheticpeptide
CRHNYGVVESFTVQR

SEQ ID NO: 7 - protein, 15 aa, synthetic construct
  REGION 1..15: note = Description of Artificial Sequence: Syntheticpeptide
TSPLTVEWRARSESA

SEQ ID NO: 8 - protein, 15 aa, synthetic construct
  REGION 1..15: note = Description of Artificial Sequence: Syntheticpeptide
FNGTERVRYLDRYFH

SEQ ID NO: 9 - protein, 15 aa, synthetic construct
  REGION 1..15: note = Description of Artificial Sequence: Syntheticpeptide
LVCSVSGFYPGSIEV

SEQ ID NO: 10 - protein, 15 aa, synthetic construct
  REGION 1..15: note = Description of Artificial Sequence: Syntheticpeptide
GLFIYFRNQKGHSGL

SEQ ID NO: 11 - protein, 15 aa, synthetic construct
  REGION 1..15: note = Description of Artificial Sequence: Syntheticpeptide
LSSPLALAGDTRPRF

SEQ ID NO: 12 - protein, 15 aa, synthetic construct
  REGION 1..15: note = Description of Artificial Sequence: Syntheticpeptide
ALTVTLMVLSSPLAL

SEQ ID NO: 13 - protein, 15 aa, synthetic construct
  REGION 1..15: note = Description of Artificial Sequence: Syntheticpeptide
LQHHNLLVCSVSGFY

SEQ ID NO: 14 - protein, 15 aa, synthetic construct
  REGION 1..15: note = Description of Artificial Sequence: Syntheticpeptide
QTLVMLETVPQSGEV

SEQ ID NO: 15 - protein, 15 aa, synthetic construct
  REGION 1..15: note = Description of Artificial Sequence: Syntheticpeptide
TSPLTVEWRARSESA

SEQ ID NO: 16 - protein, 15 aa, synthetic construct
  REGION 1..15: note = Description of Artificial Sequence: Syntheticpeptide
HNQEELVRFDSDVGE

SEQ ID NO: 17 - protein, 15 aa, synthetic construct
  REGION 1..15: note = Description of Artificial Sequence: Syntheticpeptide
GAGLFIYFRNQKGPS

SEQ ID NO: 18 - protein, 15 aa, synthetic construct
  REGION 1..15: note = Description of Artificial Sequence: Syntheticpeptide
FFNGTERVRFLERYF

SEQ ID NO: 19 - protein, 15 aa, synthetic construct
  REGION 1..15: note = Description of Artificial Sequence: Syntheticpeptide
WNSQKDILEQKRAQV

SEQ ID NO: 20 - protein, 15 aa, synthetic construct
  REGION 1..15: note = Description of Artificial Sequence: Syntheticpeptide
ALTVTLMVLSSPLAL

SEQ ID NO: 21 - protein, 15 aa, synthetic construct
  REGION 1..15: note = Description of Artificial Sequence: Syntheticpeptide
QTLVMLETVPRSGEV

SEQ ID NO: 22 - protein, 15 aa, synthetic construct
  REGION 1..15: note = Description of Artificial Sequence: Syntheticpeptide
AGLFIYFRNQKGHSG

SEQ ID NO: 23 - protein, 15 aa, synthetic construct
  REGION 1..15: note = Description of Artificial Sequence: Syntheticpeptide
FYHQEEYVRFDSDVG

SEQ ID NO: 24 - protein, 15 aa, synthetic construct
  REGION 1..15: note = Description of Artificial Sequence: Syntheticpeptide
GGFVLGLLFLGAGLF

SEQ ID NO: 25 - protein, 15 aa, synthetic construct
  REGION 1..15: note = Description of Artificial Sequence: Syntheticpeptide
RHNYGVGESFTVQRR

SEQ ID NO: 26 - protein, 15 aa, synthetic construct
  REGION 1..15: note = Description of Artificial Sequence: Syntheticpeptide
IYFRNQKGHSGLQPT

SEQ ID NO: 27 - protein, 15 aa, synthetic construct
  REGION 1..15: note = Description of Artificial Sequence: Syntheticpeptide
EYVRFDSDVGEYRAV

SEQ ID NO: 28 - protein, 15 aa, synthetic construct
  REGION 1..15: note = Description of Artificial Sequence: Syntheticpeptide
LSSPLALAGDTRPRF

SEQ ID NO: 29 - protein, 15 aa, synthetic construct
  REGION 1..15: note = Description of Artificial Sequence: Syntheticpeptide
ALTVTLMVLSSPLAL

SEQ ID NO: 30 - protein, 15 aa, synthetic construct
  REGION 1..15: note = Description of Artificial Sequence: Syntheticpeptide
QKDILEDQRASVDTF

SEQ ID NO: 31 - protein, 15 aa, synthetic construct
  REGION 1..15: note = Description of Artificial Sequence: Syntheticpeptide
LQHHTLLVCSVNGFY

SEQ ID NO: 32 - protein, 15 aa, synthetic construct
  REGION 1..15: note = Description of Artificial Sequence: Syntheticpeptide
QTLVMLETVPQSGEV

SEQ ID NO: 33 - protein, 15 aa, synthetic construct
  REGION 1..15: note = Description of Artificial Sequence: Syntheticpeptide
TSPLTVEWRARSESA

SEQ ID NO: 34 - protein, 15 aa, synthetic construct
  REGION 1..15: note = Description of Artificial Sequence: Syntheticpeptide
GAGLFIYFRNQKGHS

SEQ ID NO: 35 - protein, 15 aa, synthetic construct
  REGION 1..15: note = Description of Artificial Sequence: Syntheticpeptide
LSSPLALAGDTRPRF

SEQ ID NO: 36 - protein, 15 aa, synthetic construct
  REGION 1..15: note = Description of Artificial Sequence: Syntheticpeptide
ALTVTLMVLSSPLAL

SEQ ID NO: 37 - protein, 15 aa, synthetic construct
  REGION 1..15: note = Description of Artificial Sequence: Syntheticpeptide
LQHHNLLVCSVSGFY

SEQ ID NO: 38 - protein, 15 aa, synthetic construct
  REGION 1..15: note = Description of Artificial Sequence: Syntheticpeptide
QTLVMLETVPQSGEV

SEQ ID NO: 39 - protein, 15 aa, synthetic construct
  REGION 1..15: note = Description of Artificial Sequence: Syntheticpeptide
TSPLTVEWRARSESA

SEQ ID NO: 40 - protein, 15 aa, synthetic construct
  REGION 1..15: note = Description of Artificial Sequence: Syntheticpeptide
HNQEELVRFDSDVGE

SEQ ID NO: 41 - protein, 15 aa, synthetic construct
  REGION 1..15: note = Description of Artificial Sequence: Syntheticpeptide
GAGLFIYFRNQKGPS

SEQ ID NO: 42 - protein, 15 aa, synthetic construct
  REGION 1..15: note = Description of Artificial Sequence: Syntheticpeptide
FFNGTERVRFLERYF

SEQ ID NO: 43 - protein, 15 aa, synthetic construct
  REGION 1..15: note = Description of Artificial Sequence: Syntheticpeptide
WNSQKDILEQKRAQV

SEQ ID NO: 44 - protein, 15 aa, synthetic construct
  REGION 1..15: note = Description of Artificial Sequence: Syntheticpeptide
TRPRFLEQAKSECHF

SEQ ID NO: 45 - DNA, 20 bp, synthetic construct
  misc_feature 1..20: note = Description of Artificial Sequence: Syntheticprimer
  source 1..20: mol_type = other DNA
cgcctagagaagaggctgtg

SEQ ID NO: 46 - DNA, 20 bp, synthetic construct
  misc_feature 1..20: note = Description of Artificial Sequence: Syntheticprimer
  source 1..20: mol_type = other DNA
ctgctgtggctgtggtgtag

SEQ ID NO: 47 - protein, 15 aa, synthetic construct
  REGION 1..15: note = Description of Artificial Sequence: Syntheticpeptide
TQFVRFDSDAASQRM